European Patent Application EP 4 353 827 A2, published April 17, 2024. Title: CORYNEBACTERIUM GLUTAMICUM MUTANT STRAIN HAVING ENHANCED L-LYSINE PRODUCTIVITY AND METHOD OF PRODUCING L-LYSINE USING THE SAME. Applicant: DAESANG CORPORATION. The sequence listing filed with the application follows.

SEQUENCE LISTING (15 sequences)

SEQ ID NO: 1 - DNA, 247 bp, synthetic construct
  misc_feature 1..247: note = Promoter sequence of pyc gene
  source 1..247: mol_type = other DNA
aaatgcgttaaacttggccaaatgtggcaacctttgcaaggtgaaaaactggggcggggttagatcctggggggtttatttcattcactttggcttgaagtcgtgcaggtcaggggagtgttgcccgaaaacattgagaggaaaacaaaaaccgatgtttgattgggggaatcgggggttacgatactaggacgcagtgactgctatcacccttggcggtctcttgttgaaaggaataattactcta

SEQ ID NO: 2 - DNA, 247 bp, synthetic construct
  misc_feature 1..247: note = Mutant promoter sequence of pyc gene
  source 1..247: mol_type = other DNA
aaatgcgttaaacttggccaaatgtggcaacctttgcaaggtgaaaaactggggcggggttagatcctggggggtttatttcattcactttggcttgaagtcgtgcaggtcaggggagtgttgcccgaaaacattgagaggaaaacaaaaaccgatgtttgattgggggaatcgtgtggtatgatggtaggacgcaacagctgctactgtccttggcggtctcttgttgaaaggaataattactcta

SEQ ID NO: 3 - DNA, 247 bp, synthetic construct
  misc_feature 1..247: note = Mutant promoter sequence of pyc gene
  source 1..247: mol_type = other DNA
aaatgcgttaaacttggccaaatgtggcaacctttgcaaggtgaaaaactggggcggggttagatcctggggggtttatttcattcactttggcttgaagtcgtgcaggtcaggggagtgttgcccgaaaacattgagaggaaaacaaaaaccgatgtttgattgggggaatcgtgttgtatgattgtaggacgcaactgctgctactacccttggcggtctcttgttgaaaggaataattactcta

SEQ ID NO: 4 - DNA, 33 bp, synthetic construct
  misc_feature 1..33: note = pycP-F1
  source 1..33: mol_type = other DNA
catgtatcacgcactcggtgaaggcgtgagccc

SEQ ID NO: 5 - DNA, 55 bp, synthetic construct
  misc_feature 1..55: note = pycP-R1
  source 1..55: mol_type = other DNA
gaccgccaaggacagtagcagctgttgcgtcctaccatcataccacacgattccc

SEQ ID NO: 6 - DNA, 55 bp, synthetic construct
  misc_feature 1..55: note = pycP-F2
  source 1..55: mol_type = other DNA
gggaatcgtgtggtatgatggtaggacgcaacagctgctactgtccttggcggtc

SEQ ID NO: 7 - DNA, 33 bp, synthetic construct
  misc_feature 1..33: note = pycP-R2
  source 1..33: mol_type = other DNA
aacttctccagtgtgatcgccaaggatctgcac

SEQ ID NO: 8 - DNA, 30 bp, synthetic construct
  misc_feature 1..30: note = pycP-F3
  source 1..30: mol_type = other DNA
tgattacgcccatgtatcacgcactcggtg

SEQ ID NO: 9 - DNA, 26 bp, synthetic construct
  misc_feature 1..26: note = pycP-R3
  source 1..26: mol_type = other DNA
gtgtgatcgccaaggatctgcacttc

SEQ ID NO: 10 - DNA, 20 bp, synthetic construct
  misc_feature 1..20: note = pCGI-F1
  source 1..20: mol_type = other DNA
actggccgtcgttttacaac

SEQ ID NO: 11 - DNA, 20 bp, synthetic construct
  misc_feature 1..20: note = pCGI-R1
  source 1..20: mol_type = other DNA
ggcgtaatcatggtcatagc

SEQ ID NO: 12 - DNA, 30 bp, synthetic construct
  misc_feature 1..30: note = pCGI(pyc)-F2
  source 1..30: mol_type = other DNA
tggagaagttactggccgtcgttttacaac

SEQ ID NO: 13 - DNA, 21 bp, synthetic construct
  misc_feature 1..21: note = pCGI-R2
  source 1..21: mol_type = other DNA
tggtcatagctgtttcctgtg

SEQ ID NO: 14 - DNA, 55 bp, synthetic construct
  misc_feature 1..55: note = pycP-R4
  source 1..55: mol_type = other DNA
gaccgccaagggtagtagcagcagttgcgtcctacaatcatacaacacgattccc

SEQ ID NO: 15 - DNA, 55 bp, synthetic construct
  misc_feature 1..55: note = pycP-F4
  source 1..55: mol_type = other DNA
gggaatcgtgttgtatgattgtaggacgcaactgctgctactacccttggcggtc